European Patent Application EP 4 393 507 A1, published July 3, 2024. Title: Pharmaceutical Composition for Treatment of Peripheral Nerve Injury. Applicant: NATIONAL UNIVERSITY CORPORATION HOKKAIDO UNIVERSITY. The sequence listing filed with the application follows.

SEQUENCE LISTING (1 sequence)

SEQ ID NO: 1 - protein, 15 aa, Artificial Sequence
  Peptide moiety of PA-dPEG24
IALILEPICCQERAA